European Patent Specification EP 3 335 725 B1, published February 28, 2024. Title: Immunity inducing agent. Applicant: TORAY INDUSTRIES, INC. The sequence listing filed with the application follows.

SEQUENCE LISTING (85 sequences)

SEQ ID NO: 1 - DNA, 7190 bp, Homo sapiens
  CDS (541)..(4554)
ggccggcggaggaaggggagggagcgaggagcgcgcgctgctctcgcgtgctctcgcgccgctcgcgtgaccggccggtgtgtgcgcgaggccccggctcccggggcacggacggccgggcgcgcgcctctgcgaggggcgtccgggtccgagtcggcggtccgggccggcgcgaggtgcgtgcgggcgggccgcgggggtcccggacggacacaagcgcacacactcccggaggagccttcgaggctgctcttcctcggccagacggagagcggcactgtctccccgcccagcgctcactcgccccgcgtctccccccgcggcggctgctcctcctcggcaccgccagccccagcgccgctcccgggcgggcgggcggcggcggcggcggcggcgggacccgcggagccgctttgtgtgcagcccgactaggggcggcggcgcaaccacctgacagaggcccgggcgctcgatgcaccttccgcccgcatgaggaggagaggccggtagaggactgtgaaccaaaagttgtcccccaggatggacttcaccgcgcagcccaagcctgccactgccctctgtggcgtcgtgagtgccgacgggaagatcgcttaccctccgggggtaaaagagatcaccgacaagatcaccacggacgagatgatcaaacgcctgaagatggtagtgaaaacctttatggatatggatcaggactcagaagatgaaaaacagcagtatctcccactagccttgcatcttgcatctgaattcttcctcaggaaccccaataaagatgtgcgtctccttgtagcatgttgtttggctgatatctttcgtatctatgccccagaagctccatatacttcccatgataaacttaaggacatatttttgtttattaccagacaattaaaaggtttggaggatacaaagagtccacagtttaatagatacttttatttattagagaatttagcttgggttaaatcatataacatctgctttgaattggaagattgcaatgaaatttttattcagctttttagaactctcttctcagtgatcaacaatagccacaataagaaggtacaaatgcacatgctagatttgatgagttctatcatcatggaaggtgatggagttactcaagaattattggactccattcttattaacctcattcctgcacataagaacttaaataaacagtcctttgaccttgcaaaagtgctattgaaaagaacagtccagactattgaggcatgcattgctaattttttcaatcaagtcctggtgctgggaagatcatcagtaagtgatttgtcagaacatgtatttgatctgattcaggaactttttgctatagatcctcatttattattatccgtcatgccacagcttgaattcaaactaaagagcaatgatggagaagagcgattagctgttgttcgacttctagctaaattgtttggctccaaagattctgatttggcaacacagaatcgtcctctttggcaatgttttcttggacgatttaatgatattcatgttcctgtgagattagaaagtgtgaaatttgccagtcattgtttaatgaatcacccagatttagcgaaggatctcacagaatatttaaaggttagatcacatgatccagaagaagctattcgtcatgatgtcattgttactataataacagctgccaagagggacctggccttagtaaatgatcagctgcttggctttgtaagggaaagaacactggataaacggtggcgagtaagaaaagaagctatgatgggtctggctcagctttataagaaatactgtcttcatggtgaagcaggaaaggaagctgcagagaaagtcagctggataaaggacaaacttctgcatatttattatcagaacagcattgacgacaaactgttggtagagaaaatctttgctcagtatcttgtcccccacaacctggaaacagaagagagaatgaaatgcttatattacttatatgctagtttggatccaaatgctgtaaaagctctcaacgaaatgtggaagtgtcagaacatgcttcggagccatgtacgcgaactattggatttgcacaagcagcctacatcagaggctaactgttctgccatgtttggaaaactgatgaccatagcaaagaatttgcctgaccccgggaaagcacaagattttgtgaagaaatttaaccaggttctcggcgatgatgagaaacttcggtctcagttggagttattaattagcccaacctgttcttgcaaacaagcagatatttgtgtgagagaaatagcccggaaacttgcaaatcctaagcaaccaacaaatccttttctagagatggtcaaatttctgttggaaagaatcgcacctgtgcacattgattcagaagccataagtgcactagtgaaattgatgaataagtcaatagaggggacagcagatgatgaagaggagggtgtaagtccagatacagctatccgttcaggacttgaacttcttaaggttctgtcttttacacatcctacctcgttccactctgcagagacatatgagtccttgttacagtgcctaagaatggaggatgacaaggtagcagaagctgctattcaaatttttagaaatacaggtcacaaaatagaaacagaccttccccagatacgatcgaccttaattcccattttacatcaaaaagcaaagaggggtactccacaccaagcaaaacaggctgtgcactgtatacacgccatattcacaaataaagaagtccagcttgcacagatttttgagccactcagtaggagtctgaatgctgatgtgccagaacaacttataactccattagtttcattgggccacatttctatgttagcaccagatcagtttgcttccccaatgaaatctgtagtagcaaattttattgtgaaagatctgctaatgaatgacaggtcaacaggtgaaaagaatggaaaactgtggtctccagatgaagaggtttcccctgaagtactagcaaaggtacaggcaattaaacttctggtaaggtggctgttgggtatgaaaaacaaccagtctaaatctgccaattcaacccttcggttattatcagcgatgttggttagtgagggtgacctgacagagcaaaagaggatcagtaaatctgatatgtctcgcttgcgattagctgctggtagtgccataatgaagcttgctcaggaaccttgttaccatgaaattattaccccagaacagtttcagctctgtgcacttgttattaatgatgagtgttaccaagtaaggcagatatttgctcagaagctgcataaggcacttgtgaagttactgctcccattggagtatatggcgatctttgccttgtgtgccaaagatcctgtgaaggagagaagagcacacgcacgacaatgtttactgaaaaatatcagtatacgcagggaatacattaagcagaatcctatggctactgagaaattattatcactgttgcctgaatatgtagttccatacatgattcacctgctagcccatgatccagattttacaagatcacaagatgttgatcagcttcgtgatatcaaagagtgcctatggttcatgcttgaagttttaatgacaaagaatgaaaacaatagccatgcctttatgaagaagatggcagagaacatcaagttaaccagagatgcccagtctccagatgaatccaagacaaatgaaaaactgtatacagtatgtgatgtggctctctgtgttataaatagtaaaagtgctttgtgcaatgcagattcaccaaaggacccagtcctcccaatgaaattttttacacaacctgaaaaggacttctgtaacgataagagttatatttcagaagagacaagagtacttctgttaacaggaaagccaaagcctgctggagtactaggtgcagtaaataagcctttatcagcaacgggaaggaaaccctatgttagaagcactggcactgagactggaagcaatattaatgtaaattcagagctgaacccttcaaccggaaatcgatcaagggaacagagttcagaggcagcagaaactggagttagtgaaaatgaagagaaccctgtgaggattatttcagtcacacctgtaaagaatattgacccagtaaagaataaggaaattaattctgatcaggctacccagggcaacatcagcagtgaccgaggaaagaaaagaacagtaacagcagctggtgcagagaatatccaacaaaaaacagatgagaaagtagatgaatcgggacctcccgccccttccaaacccaggagaggacgtcgacccaagtctgaatctcagggcaatgctaccaaaaatgatgatctaaataaacctattaacaagggaaggaagagagctgcagtgggtcaggagagccctgggggtttggaagcaggtaatgccaaagcacccaaactgcaagatttagccaaaaaggcagcaccagcagaaagacaaattgacttacaaaggtaaaaatgcatttgcaaagggagaaaatgaaggccaaacagaagcaggctccagcttctgcaaaaacttggattcacaaatgtccctgaacagaaaatgaagctcacttcagaacacacactctctgccttgaaaactaaagagactattacttccttttcacatgaccacaagtcctctgatggaaatgtacagcagaaactcttgagagagaggctaaaagcaactctgttctcccccttcccctagacttttcttacgaaaagtcaataattaagcaaattgcttaacacttggttccagttcctgcctatctggagtttaaatgcgtaatacaccattaatttccacgctgcagtttttattttaaagaaagtaacaagatgtctttacactgacactgaaaattcatccattttagagccaggaattcccatgttacacaggaaaaaatagaagtctactgaattaattttttaaaagaaaagagatcagattaaatatttctttgtttttccttttggaaacttttatgtataattctttctgcctgcctacttttctgcaaaaatgagatgtacagatttcggttccctgctatgaaaagtgatgtggtagcaattttataaatgttgctttctgatttttatcagagtgagaaaattaaaattattgatttgcaagtagtaaacagttcatattttgatttcccctcattttagtttaatataatttgcaataaatgtacatattgttgtttgtttcataaagcatatcactttaaaatggtttttactcctgtgattatgttggaatatttggaattttaaaggagtaaagactgtccagcatttggttttataatgtttgtcaccagatttttattaatgtaaaaaaaatcaatttttaaaaaatagttggactttggcagcttttaaggaaagttggaggtgttttaggattgctatcaattttcagcattgtgctatttggaaataagtgttttgcttttgtctgatggtctgggctcatttttatgtttattttagaaaactgttgcatcaatatattatgtttcttggcattgttcagcataggtaatgtgtgcactttatgtgtacacataatcatatttaagttttttgcataaaataaatgcttctagatgtcatggcagtctttttaatctttttatcatatgctttcttgtgaattttttcatgttaaagagctaaagtcataacatgattacagtcaactctccattatctatataaaatagtgactaagcctcaggtttttaattttgtgataacaaaataacgaaggcatgtaagacctgattctggaggaacatgaaatttgtcttttctcatgtccagagttctatcctgcccccactgtccactgtagggtcatccgcaaagccctagcagaatgtgctcactccatttccttacacgtttctagcatgggtcagaggaaacaacatttgtgttataacttcgtcttgataggctgtagtgtacatgggatgtaaaacaaacaagtgtatcaaaggtggatgattctgttagagtgaagtttgagagtaaatgtcacttacgtttctcatagataatcaagagttggctgtgtattgactgaaagatgggtaattattttaaatatgcatttacacacatttaggtatcagaagatgcttagggaacaatggataccaatgatagaaaatgatacctttacaggggcagaaaaatccccactcttccttattgcctcttcagaaccctttagaaagtataaaatattgcctccaacatgctgaaaaagagtatctatgcataagtatcagagaagtccctcaagcaatcagtaggtgtgttctatttagagagagtttaaagttctcttagcatcagacaacttgattcctaaggtttccagtgtgtcaccaacaaaaagtgcattgatagggacctttgtctcttcctccctttgattaattgcccggcatcacagtttactagattaccaagtgttacatcatattaaataaaatgtagcagaaccatctgcatcaatatattcctgtttagatttttgcaggagagaagttaaaaggatttgctccttgtatgatgtaagtggcccaccccaattttgtaacatgatgcaagtgtctggcactaagggaagcaagagtagggttgtggaaagaccaagctgatggggagggacttgtttacgggaatttttttagttttccttttcaaaggaaaacattaaaatcccttaggaatttggtattcacatctcagagaactacaacacaaaagtgcagacttatatttgagaattaatgttaaccctttgtgtctagtttgaagcttcttgtatttgtctaaaacaacaagccagaattttgtatctcctttgataaaaagtgtgtataatgtaaagtagttttgcatattcttgtgctgcacatgggctgaatttttaaattttttttaaaaacttgaagcagaaccttgtaatttgtgtaaatgacaagtgtaaaatcctaccataaaatgctaaaaatatgcactgtttcaaataaaaccaagaaatgcagcattaaaaaaaaaaaaaaa

SEQ ID NO: 2 - protein, 1337 aa, Homo sapiens
MDFTAQPKPATALCGVVSADGKIAYPPGVKEITDKITTDEMIKRLKMVVKTFMDMDQDSEDEKQQYLPLALHLASEFFLRNPNKDVRLLVACCLADIFRIYAPEAPYTSHDKLKDIFLFITRQLKGLEDTKSPQFNRYFYLLENLAWVKSYNICFELEDCNEIFIQLFRTLFSVINNSHNKKVQMHMLDLMSSIIMEGDGVTQELLDSILINLIPAHKNLNKQSFDLAKVLLKRTVQTIEACIANFFNQVLVLGRSSVSDLSEHVFDLIQELFAIDPHLLLSVMPQLEFKLKSNDGEERLAVVRLLAKLFGSKDSDLATQNRPLWQCFLGRFNDIHVPVRLESVKFASHCLMNHPDLAKDLTEYLKVRSHDPEEAIRHDVIVTIITAAKRDLALVNDQLLGFVRERTLDKRWRVRKEAMMGLAQLYKKYCLHGEAGKEAAEKVSWIKDKLLHIYYQNSIDDKLLVEKIFAQYLVPHNLETEERMKCLYYLYASLDPNAVKALNEMWKCQNMLRSHVRELLDLHKQPTSEANCSAMFGKLMTIAKNLPDPGKAQDFVKKFNQVLGDDEKLRSQLELLISPTCSCKQADICVREIARKLANPKQPTNPFLEMVKFLLERIAPVHIDSEAISALVKLMNKSIEGTADDEEEGVSPDTAIRSGLELLKVLSFTHPTSFHSAETYESLLQCLRMEDDKVAEAAIQIFRNTGHKIETDLPQIRSTLIPILHQKAKRGTPHQAKQAVHCIHAIFTNKEVQLAQIFEPLSRSLNADVPEQLITPLVSLGHISMLAPDQFASPMKSVVANFIVKDLLMNDRSTGEKNGKLWSPDEEVSPEVLAKVQAIKLLVRWLLGMKNNQSKSANSTLRLLSAMLVSEGDLTEQKRISKSDMSRLRLAAGSAIMKLAQEPCYHEIITPEQFQLCALVINDECYQVRQIFAQKLHKALVKLLLPLEYMAIFALCAKDPVKERRAHARQCLLKNISIRREYIKQNPMATEKLLSLLPEYVVPYMIHLLAHDPDFTRSQDVDQLRDIKECLWFMLEVLMTKNENNSHAFMKKMAENIKLTRDAQSPDESKTNEKLYTVCDVALCVINSKSALCNADSPKDPVLPMKFFTQPEKDFCNDKSYISEETRVLLLTGKPKPAGVLGAVNKPLSATGRKPYVRSTGTETGSNINVNSELNPSTGNRSREQSSEAAETGVSENEENPVRIISVTPVKNIDPVKNKEINSDQATQGNISSDRGKKRTVTAAGAENIQQKTDEKVDESGPPAPSKPRRGRRPKSESQGNATKNDDLNKPINKGRKRAAVGQESPGGLEAGNAKAPKLQDLAKKAAPAERQIDLQR

SEQ ID NO: 3 - protein, 9 aa, Homo sapiens
YLPLALHLA

SEQ ID NO: 4 - protein, 10 aa, Homo sapiens
LLVACCLADI

SEQ ID NO: 5 - protein, 9 aa, Homo sapiens
YLLENLAWV

SEQ ID NO: 6 - protein, 9 aa, Homo sapiens
QLFRTLFSV

SEQ ID NO: 7 - protein, 9 aa, Homo sapiens
LLDSILINL

SEQ ID NO: 8 - protein, 10 aa, Homo sapiens
AIDPHLLLSV

SEQ ID NO: 9 - protein, 9 aa, Homo sapiens
YLVPHNLET

SEQ ID NO: 10 - protein, 10 aa, Homo sapiens
YLYASLDPNA

SEQ ID NO: 11 - protein, 9 aa, Homo sapiens
AMFGKLMTI

SEQ ID NO: 12 - protein, 9 aa, Homo sapiens
FLLERIAPV

SEQ ID NO: 13 - protein, 9 aa, Homo sapiens
LNADVPEQL

SEQ ID NO: 14 - protein, 8 aa, Homo sapiens
QLITPLVS

SEQ ID NO: 15 - protein, 10 aa, Homo sapiens
KLWSPDEEVS

SEQ ID NO: 16 - protein, 9 aa, Homo sapiens
VINDECYQV

SEQ ID NO: 17 - protein, 9 aa, Homo sapiens
YMAIFALCA

SEQ ID NO: 18 - protein, 10 aa, Homo sapiens
KLYTVCDVAL

SEQ ID NO: 19 - protein, 10 aa, Homo sapiens
YTVCDVALCV

SEQ ID NO: 20 - protein, 9 aa, Homo sapiens
AYPPGVKEI

SEQ ID NO: 21 - protein, 9 aa, Homo sapiens
QYLPLALHL

SEQ ID NO: 22 - protein, 9 aa, Homo sapiens
IFLFITRQL

SEQ ID NO: 23 - protein, 9 aa, Homo sapiens
QFNRYFYLL

SEQ ID NO: 24 - protein, 9 aa, Homo sapiens
RYFYLLENL

SEQ ID NO: 25 - protein, 9 aa, Homo sapiens
FYLLENLAW

SEQ ID NO: 26 - protein, 10 aa, Homo sapiens
AWVKSYNICF

SEQ ID NO: 27 - protein, 9 aa, Homo sapiens
IFIQLFRTL

SEQ ID NO: 28 - protein, 9 aa, Homo sapiens
VFDLIQELF

SEQ ID NO: 29 - protein, 9 aa, Homo sapiens
LFAIDPHLL

SEQ ID NO: 30 - protein, 9 aa, Homo sapiens
LWQCFLGRF

SEQ ID NO: 31 - protein, 10 aa, Homo sapiens
YYQNSIDDKL

SEQ ID NO: 32 - protein, 9 aa, Homo sapiens
TYESLLQCL

SEQ ID NO: 33 - protein, 9 aa, Homo sapiens
IFRNTGHKI

SEQ ID NO: 34 - protein, 9 aa, Homo sapiens
IFEPLSRSL

SEQ ID NO: 35 - protein, 16 aa, Homo sapiens
ASEFFLRNPNKDVRLL

SEQ ID NO: 36 - protein, 19 aa, Homo sapiens
LKDIFLFITRQLKGLEDTK

SEQ ID NO: 37 - protein, 17 aa, Homo sapiens
FNRYFYLLENLAWVKSY

SEQ ID NO: 38 - protein, 15 aa, Homo sapiens
NLAWVKSYNICFELE

SEQ ID NO: 39 - protein, 18 aa, Homo sapiens
NEIFIQLFRTLFSVINNS

SEQ ID NO: 40 - protein, 17 aa, Homo sapiens
TLFSVINNSHNKKVQMH

SEQ ID NO: 41 - protein, 18 aa, Homo sapiens
NKKVQMHMLDLMSSIIME

SEQ ID NO: 42 - protein, 19 aa, Homo sapiens
LDSILINLIPAHKNLNKQS

SEQ ID NO: 43 - protein, 23 aa, Homo sapiens
IQELFAIDPHLLLSVMPQLEFKL

SEQ ID NO: 44 - protein, 18 aa, Homo sapiens
GEERLAVVRLLAKLFGSK

SEQ ID NO: 45 - protein, 19 aa, Homo sapiens
HDVIVTIITAAKRDLALVN

SEQ ID NO: 46 - protein, 19 aa, Homo sapiens
SAMFGKLMTIAKNLPDPGK

SEQ ID NO: 47 - protein, 16 aa, Homo sapiens
AQDFVKKFNQVLGDDE

SEQ ID NO: 48 - protein, 21 aa, Homo sapiens
IDSEAISALVKLMNKSIEGTA

SEQ ID NO: 49 - protein, 15 aa, Homo sapiens
PTSFHSAETYESLLQ

SEQ ID NO: 50 - protein, 18 aa, Homo sapiens
EAAIQIFRNTGHKIETDL

SEQ ID NO: 51 - protein, 18 aa, Homo sapiens
LPQIRSTLIPILHQKAKR

SEQ ID NO: 52 - protein, 16 aa, Homo sapiens
LIPILHQKAKRGTPHQ

SEQ ID NO: 53 - protein, 20 aa, Homo sapiens
KQAVHCIHAIFTNKEVQLAQ

SEQ ID NO: 54 - protein, 15 aa, Homo sapiens
ASPMKSVVANFIVKD

SEQ ID NO: 55 - protein, 19 aa, Homo sapiens
VLAKVQAIKLLVRWLLGMK

SEQ ID NO: 56 - protein, 18 aa, Homo sapiens
KLLVRWLLGMKNNQSKSA

SEQ ID NO: 57 - protein, 20 aa, Homo sapiens
SANSTLRLLSAMLVSEGDLT

SEQ ID NO: 58 - protein, 18 aa, Homo sapiens
KSDMSRLRLAAGSAIMKL

SEQ ID NO: 59 - protein, 19 aa, Homo sapiens
CYQVRQIFAQKLHKALVKL

SEQ ID NO: 60 - protein, 15 aa, Homo sapiens
PLEYMAIFALCAKDP

SEQ ID NO: 61 - protein, 18 aa, Homo sapiens
AHARQCLLKNISIRREYI

SEQ ID NO: 62 - protein, 15 aa, Homo sapiens
RREYIKQNPMATEKL

SEQ ID NO: 63 - protein, 22 aa, Homo sapiens
ECLWFMLEVLMTKNENNSHAFM

SEQ ID NO: 64 - protein, 23 aa, Homo sapiens
SHAFMKKMAENIKLTRDAQSPDE

SEQ ID NO: 65 - protein, 23 aa, Homo sapiens
KSYISEETRVLLLTGKPKPAGVL

SEQ ID NO: 66 - protein, 18 aa, Homo sapiens
PAGVLGAVNKPLSATGRK

SEQ ID NO: 67 - protein, 17 aa, Homo sapiens
ENPVRIISVTPVKNIDP

SEQ ID NO: 68 - DNA, 21 bp, Artificial
  primer sense
gtaaggtggctgttgggtatg

SEQ ID NO: 69 - DNA, 24 bp, Artificial
  primer antisense
ggctagcaggtgaatcatgtatgg

SEQ ID NO: 70 - DNA, 18 bp, Artificial
  GAPDH primer
gggctgcttttaactctg

SEQ ID NO: 71 - DNA, 18 bp, Artificial
  GAPDH primer
ccaggaaatgagcttgac

SEQ ID NO: 72 - DNA, 29 bp, Artificial
  primer sense
gcggccgcatggacttcaccgcgcagccc

SEQ ID NO: 73 - DNA, 29 bp, Artificial
  primer antisense
ctcgagttacctttgtaagtcaatttgtc

SEQ ID NO: 74 - protein, 9 aa, Homo sapiens
SLYNTYATL

SEQ ID NO: 75 - protein, 9 aa, Homo sapiens
NLIPAHKNL

SEQ ID NO: 76 - protein, 10 aa, Homo sapiens
KECLWFMLEV

SEQ ID NO: 77 - protein, 10 aa, Homo sapiens
FLGRFNDIHV

SEQ ID NO: 78 - protein, 10 aa, Homo sapiens
LLLPLEYMAI

SEQ ID NO: 79 - protein, 10 aa, Homo sapiens
SLDPNAVKAL

SEQ ID NO: 80 - protein, 9 aa, Homo sapiens
KLKDIFLFI

SEQ ID NO: 81 - protein, 10 aa, Homo sapiens
LLSLLPEYVV

SEQ ID NO: 82 - protein, 9 aa, Homo sapiens
KMAENIKLT

SEQ ID NO: 83 - protein, 10 aa, Homo sapiens
QVLVLGRSSV

SEQ ID NO: 84 - protein, 9 aa, Homo sapiens
RYLRDQQLL

SEQ ID NO: 85 - protein, 18 aa, Homo sapiens
YVDRFFKTLRAEQATQDV